European Patent Application EP 4 707 410 A2, published March 11, 2026. Title: REGULATE GUT MICROBIOTA TO TREAT NEURODEGENERATIVE DISORDERS. Applicant: California Institute of Technology. Application EP. The sequence listing filed with the application follows.

SEQUENCE LISTING (12 sequences)

SEQ ID NO: 1 - DNA, 21 bp, synthetic construct
  misc_feature 1..21: note = Synthetic oligonucleotide
  source 1..21: mol_type = other DNA
ttgcagcagccactggctttg

SEQ ID NO: 2 - DNA, 25 bp, synthetic construct
  misc_feature 1..25: note = Synthetic oligonucleotide
  source 1..25: mol_type = other DNA
ggatccacaggcatatcttccagaa

SEQ ID NO: 3 - DNA, 23 bp, synthetic construct
  misc_feature 1..23: note = Synthetic oligonucleotide
  source 1..23: mol_type = other DNA
ccctcacactcagatcatcttct

SEQ ID NO: 4 - DNA, 19 bp, synthetic construct
  misc_feature 1..19: note = Synthetic oligonucleotide
  source 1..19: mol_type = other DNA
gctacgacgtgggctacag

SEQ ID NO: 5 - DNA, 23 bp, synthetic construct
  misc_feature 1..23: note = Synthetic oligonucleotide
  source 1..23: mol_type = other DNA
tagtccttcctaccccaatttcc

SEQ ID NO: 6 - DNA, 21 bp, synthetic construct
  misc_feature 1..21: note = Synthetic oligonucleotide
  source 1..21: mol_type = other DNA
ttggtccttagccactccttc

SEQ ID NO: 7 - DNA, 20 bp, synthetic construct
  misc_feature 1..20: note = Synthetic oligonucleotide
  source 1..20: mol_type = other DNA
caaggcaagagctgccatag

SEQ ID NO: 8 - DNA, 19 bp, synthetic construct
  misc_feature 1..19: note = Synthetic oligonucleotide
  source 1..19: mol_type = other DNA
ccggtacttagcgtcaggg

SEQ ID NO: 9 - DNA, 22 bp, synthetic construct
  misc_feature 1..22: note = Synthetic oligonucleotide
  source 1..22: mol_type = other DNA
tcatacttcggttgcatgaagg

SEQ ID NO: 10 - DNA, 19 bp, synthetic construct
  misc_feature 1..19: note = Synthetic oligonucleotide
  source 1..19: mol_type = other DNA
agacctctcgaacctgccc

SEQ ID NO: 11 - DNA, 20 bp, synthetic construct
  misc_feature 1..20: note = Synthetic oligonucleotide
  source 1..20: mol_type = other DNA
catggccttccgtgttccta

SEQ ID NO: 12 - DNA, 22 bp, synthetic construct
  misc_feature 1..22: note = Synthetic oligonucleotide
  source 1..22: mol_type = other DNA
cctgcttcaccaccttcttgat